European Patent Application EP 4 560 014 A1, published May 28, 2025. Title: 닭전염성기관지염바이러스 약독화주 및 이를 포함하는 백신조성물. Applicant: 주식회사 카브. The sequence listing filed with the application follows.

SEQUENCE LISTING (6 sequences)

SEQ ID NO: 1 - DNA, 20 bp, synthetic construct
  source 1..20: mol_type = other DNA
tggaaaaacactgcacgcaa

SEQ ID NO: 2 - DNA, 21 bp, synthetic construct
  source 1..21: mol_type = other DNA
tcacctgaacaatcgtcagct

SEQ ID NO: 3 - DNA, 3498 bp, synthetic construct
  source 1..3498: mol_type = other DNA
atgttggggaagtcactgtttttagtgaccattttgtgtgcactatgtagtgcaaatttgtttgattctgccaataattatgtgtactactaccaaagtgcctttaggcctcctactggatggcatcttcaagggggtgcttatgcagtagtgaattctactaattacactagtaatgccggttctgcaagtgggtgcactgttggtgtcatcaaggacgtttataatcaaagtgcggcttccatagctatgacagcaccttctcagggtatggcttggtctaagtcacaattttgtagtgcacactgtaacttttctgaaattacagtttttgtcacacattgttatagtagtgctacagggtcttgtcctataacaggcctgattgcacaggatcatattcgtatttcagcaatgaaaaatggttttttattttataatttaacagttagcgtatctaaataccctagatttaagtcttttcaatgtgttaacaacttcacatctgtttatttaaatggtgatcttgtttttacttctaataaaactactgatgttacgtcagcaggtgtgtattttaaagcaggtggacctgtaaactatagtgttatgaaagaatttaaggttcttgcttactttgttaatggtacagcacaagatgtaattttgtgtgacaattcccctaagggtttgctagcttgtcaatataacactggcaatttttcagacggcttttatccttttactaatagtactttagttagggacaagttcattgtctatcgtgaaagtagtgttaatactactttgacgttaactaatttcacttttactaatgtaagtactgcacagcctaatagtggtggtgttagtacttttcatctatatcaaacacaaacagctcagagtggttattataattttaatttgtcatttctgagtcagtttgtgtataaggcaagtgattttatgtatgggtcttatcatcctaggtgttcttttagaccagaaaccattaatagtggtttatggtttaattctttgtcagtttctcttacttatggacccctacagggagggtgtaagcaatctgtttttagtggtaaggcaacgtgttgttatgcctactcttataatggccctagggcatgtaaaggtgtttattcaggtgaattaagcaagacttttgaatgtggattgctggtttatgttactaagagtgatggctctcgtatacagactagaacagagcccttagtattaacgcaacacaattataataatattactttagataagtgtgttgactataatatatatggcagagtaggccaaggttttattactaatgtgactgattctgctgctaattctagttatttagcagatggtgggttagctattttagatacttcgggtgccatagatgtctttgttgtacagggcagctatggtcttaattattacaaggttaatccttgtgaagatgttaatcaacagtttgtagtgtctggtggcaatatagttggcatccttacttctagaaatgaaacaggttctgaacaggttgagaaccagttttatgttaagttaaccaatagctcacatcgtcgtaggcgttctattggccaaaatgtaacaagttgttcttatgttagttatggcagattttgtattgaaccagatggttcgttaaagatgatagtgccagaagaattgaagcagtttgtggcacctttacttaatattactgaaagtgtactcatacctaacagttttaatttgactgttacagatgagtacatacaaacacgtatggataaggtccaaatcaattgccttcaatatgtttgcggcaattctttggagtgtagaaaattgtttcaacaatatggtccggtttgtgataacatattgtctgttgtaaatagtgttggtcaaaaagaagatatggaacttttaagtttctattcttctactaaaccagctggttataatgcacctgtttttagtaatattagtactggtgattttaatatctctcttttattaacaccacctagcagtcctagcggtcgctcttttatagaagatttgttatttacaagtgttgaaacagttggtttgccaactgatgctgaatataaaaaatgcacagcaggacctttaggtactcttaaggatcttatctgtgctagggaatataatggtttattagtgttgcctccaattattacggcggatatgcaaacaatgtatactgcttctttagttggtgccatggcttttggtggtattacagcagcaggtgccataccatttgcaactcagatacaagccagaattaatcatttgggtattacgcagtctctgttattgaaaaatcaagagaaaattgcagcttcctttaataaggccattggtcatatgcaggaaggttttagaagcacttcgctagcattacaacaggttcaagacgttgttaataagcagagtgctattcttactgaaattatgaattctcttaataagaattttggtgctatttcatcagtaattcaagacatttatgcgcaacttgatgcaattcaagcagatgcacaagtagaccgtcttattactggcagactctcttctctctcagttctagcctctgctaagcaatctgagtacatcagagtttcccaacaacgtgaattggctactcaaaaaattaatgagtgtgttaaatcacaatctaataggtatggtttttgtggtagtggaagacatgttctttcgataccacaaaatgcacctaatggtatagtgtttatacactttagttacactccagagagttttgttaatgttactgcaatagtaggtttttgtgtacagcctgctaatgctagtcagtatgcaatagtgcctgttaatggtagaggtatttttatacaagttaatggtagttactatatcactgcacgtgatatgtatatgcctagagatattactgcaggagatgtagttactcttacttcttgtcaagcaaattatgttaatgtaaataaaaccgtcattactacatttgtggaagatgacgattttgattttgatgatgagttgtcgaaatggtggaatgatactaagcatgagctaccagactttgacgacttcaattatacagtacccatacttaatattagtggtgaaattgatcatattcaaggtgttatacagggtcttaatgactcccttataaaccttgaagaactttcaatacttaaaacttatattaagtggccttggtatgtttggctagccataggctttgctattattatctttatccttattctaggatgggtgtttttcatgacaggttgttgtggttgttgttgtggatgctttggtatcattcctctaatgagtaagtgtggtaagaaatcatcttattacacgacttttgataatgatgtggtaactgaacaatacagacctaaaaagtctgtttaa

SEQ ID NO: 4 - DNA, 3471 bp, synthetic construct
  source 1..3471: mol_type = other DNA
atgttggggaagtcactgtttttagtgaccattttgtgtgcactatgtagtgcaaatttgtttgattctgccaataattatgtgtactactaccaaagtgcctttaggcctcctattggatggcatcttcaagggggtgcttatgcagtagtgaattctactaattacactagtaatgccggttctgcaagtgggtgcactgttggtgtcattaaggacgtttataatcaaagtgcggcttccatagctatgacagcaccttctcagggtatggcttggtctaagtcacaattttgtagtgcacactgtaacttttctgaaattacagtttttgtcacacattgttatagtagtgctacagggtcttgtcctataacaggcctgattgcacaggatcatattcgtatttcagcaatgaaaaatggttttttattttataatttaacagttagcgtatctaaataccctagatttaagtcttttcaatgtgttaacaacttcacatctgtttatttaaatggtgatcttgtttttacttctaataaaactactgatgttacgtcagcaggtgtgtattttaaagcaggtggacctgtaaactatagtgttatgaaagaatttaaggttcttgcttactttgttaatggtacagcacaagatgtaattttgtgtgacaattcccctaagggtttgctagcttgtcaatataacactggcaatttttcagacggcttttatccttttactaatagtactttagttagggacaagttcattgtctatcgtgaaagtagtgttaatactactttgacgttaactaatttcacttttactaatgtaagtactgcacagcctaatagtggtggtgttagtacttttcatctatatcaaacacaaacagctcagagtggttattataattttaatttgtcatttctgagtcagtttgtgtataaggcaagtgattttatgtatgggtcttatcatcctaggtgttcttttagaccagaaaccattaatagtggtttatggtttaattctttgtcagtttctcttacttatggacccctacagggagggtgtaagcaatctgtttttagtggtaaggcaacgtgttgttatgcctactcttataatggccctagggcatgtaaaggtgtttattcaggtgaattaagcaagacttttgaatgtggattgctggtttatgttactaagagtgatggctctcgtatacagactagaacagagcccttagtattaacgcaacacaattataataatattactttagataagtgtgttgactataatatatatggcagagtaggccaaggttttattactaatgtgactgattctgctgctaattctagttatttagcagatggtgggttagctattttagatacttcgggtgccatagatgtctttgttgtacagggcagctatggtcttaattattacaaggttaatccttgtgaagatgttaatcaacagtttgtagtgtctggtggcaatatagttggcatccttacttctagaaatgaaacaggttctgaacaggttgagaaccagttttatgttaagttaaccaatagctcacatcgtcgtaggcgttctattggccaaaatgtaacaagttgttcttatgttagttatggcagattttgtattgaaccagatggttcgttaaagatgatagtgccagaagaattgaagcagtttgtggcacctttacttaatattactgaaagtgtactcatacctaacagttttaatttgactgttacagatgagtacatacaaacacgtatggataaggtccaaatcaattgccttcaatatgtttgcggcaattctttggagtgtagaaaattgtttcaacaatatggtccggtttgtgataacatattgtctgttgtaaatagtgttggtcaaaaagaagatatggaacttttaagtttctattcttctactaaaccagctggttataatgcacctgtttttagtaatattagtactggtgattttaatatctctcttttattaacaccacctagcagtcctagcggtcgctcttttatagaagatttgttatttacaagtgttgaaacagttggtttgccaactgatgctgaatataaaaaatgcacagcaggacctttaggtactcttaaggatcttatctgtgctagggaatataatggtttattagtgttgcctccaattattacggcggatatgcaaacaatgtatactgcttctttagttggtgccatggcttttggtggtattacagcagcaggtgccataccatttgcaactcagatacaagccagaattaatcatttgggtattacgcagtctctgttattgaaaaatcaagagaaaattgcagcttcctttaataaggccattggtcatatgcaggaaggttttagaagcacttcgctagcattacaacaggttcaagacgttgttaataagcagagtgctattcttactgaaattatgaattctcttaataagaattttggtgctatttcatcagtaattcaagacatttatgcgcaacttgatgcaattcaagcagatgcacaagtagaccgtcttattactggcagactctcttctctctcagttctagcctctgctaagcaatctgagtacatcagagtttcccaacaacgtgaattggctactcaaaaaattaatgagtgtgttaaatcacaatctaataggtatggtttttgtggtagtggaagacatgttctttcgataccacaaaatgcacctaatggtatagtgtttatacactttagttacactccagagagttttgttaatgttactgcaatagtaggtttttgtgtacagcctgctaatgctagtcagtatgcaatagtgcctgttaatggtagaggtatttttatacaagttaatggtagttactatatcactgcacgtgatatgtatatgcctagagatattactgcaggagatgtagttactcttacttcttgtcaagcaaattatgttaatgtaaataaaaccgtcattactacatttgtggaagatgacgattttgattttgatgatgagttgtcgaaatggtggaatgatactaagcatgagctaccagactttgacgacttcaattatacagtacccatacttaatattagtggtgaaattgatcatattcaaggtgttatacagggtcttaatgactcccttataaaccttgaagaactttcaatacttaaaacttatattaagtggccttggtatgtttggctagccataggctttgctattattatctttatccttattctaggatgggtgtttttcatgacaggttgttgtggttgttgttgtggatgctttggtatcattcctctaatgagtaagtgtggtaagaaatcatcttattacacgacttttgataatgatgtggtaacttaa

SEQ ID NO: 5 - protein, 1165 aa, synthetic construct
MLGKSLFLVTILCALCSANLFDSANNYVYYYQSAFRPPTGWHLQGGAYAVVNSTNYTSNAGSASGCTVGVIKDVYNQSAASIAMTAPSQGMAWSKSQFCSAHCNFSEITVFVTHCYSSATGSCPITGLIAQDHIRISAMKNGFLFYNLTVSVSKYPRFKSFQCVNNFTSVYLNGDLVFTSNKTTDVTSAGVYFKAGGPVNYSVMKEFKVLAYFVNGTAQDVILCDNSPKGLLACQYNTGNFSDGFYPFTNSTLVRDKFIVYRESSVNTTLTLTNFTFTNVSTAQPNSGGVSTFHLYQTQTAQSGYYNFNLSFLSQFVYKASDFMYGSYHPRCSFRPETINSGLWFNSLSVSLTYGPLQGGCKQSVFSGKATCCYAYSYNGPRACKGVYSGELSKTFECGLLVYVTKSDGSRIQTRTEPLVLTQHNYNNITLDKCVDYNIYGRVGQGFITNVTDSAANSSYLADGGLAILDTSGAIDVFVVQGSYGLNYYKVNPCEDVNQQFVVSGGNIVGILTSRNETGSEQVENQFYVKLTNSSHRRRRSIGQNVTSCSYVSYGRFCIEPDGSLKMIVPEELKQFVAPLLNITESVLIPNSFNLTVTDEYIQTRMDKVQINCLQYVCGNSLECRKLFQQYGPVCDNILSVVNSVGQKEDMELLSFYSSTKPAGYNAPVFSNISTGDFNISLLLTPPSSPSGRSFIEDLLFTSVETVGLPTDAEYKKCTAGPLGTLKDLICAREYNGLLVLPPIITADMQTMYTASLVGAMAFGGITAAGAIPFATQIQARINHLGITQSLLLKNQEKIAASFNKAIGHMQEGFRSTSLALQQVQDVVNKQSAILTEIMNSLNKNFGAISSVIQDIYAQLDAIQADAQVDRLITGRLSSLSVLASAKQSEYIRVSQQRELATQKINECVKSQSNRYGFCGSGRHVLSIPQNAPNGIVFIHFSYTPESFVNVTAIVGFCVQPANASQYAIVPVNGRGIFIQVNGSYYITARDMYMPRDITAGDVVTLTSCQANYVNVNKTVITTFVEDDDFDFDDELSKWWNDTKHELPDFDDFNYTVPILNISGEIDHIQGVIQGLNDSLINLEELSILKTYIKWPWYVWLAIGFAIIIFILILGWVFFMTGCCGCCCGCFGIIPLMSKCGKKSSYYTTFDNDVVTEQYRPKKSV

SEQ ID NO: 6 - protein, 1156 aa, synthetic construct
MLGKSLFLVTILCALCSANLFDSANNYVYYYQSAFRPPIGWHLQGGAYAVVNSTNYTSNAGSASGCTVGVIKDVYNQSAASIAMTAPSQGMAWSKSQFCSAHCNFSEITVFVTHCYSSATGSCPITGLIAQDHIRISAMKNGFLFYNLTVSVSKYPRFKSFQCVNNFTSVYLNGDLVFTSNKTTDVTSAGVYFKAGGPVNYSVMKEFKVLAYFVNGTAQDVILCDNSPKGLLACQYNTGNFSDGFYPFTNSTLVRDKFIVYRESSVNTTLTLTNFTFTNVSTAQPNSGGVSTFHLYQTQTAQSGYYNFNLSFLSQFVYKASDFMYGSYHPRCSFRPETINSGLWFNSLSVSLTYGPLQGGCKQSVFSGKATCCYAYSYNGPRACKGVYSGELSKTFECGLLVYVTKSDGSRIQTRTEPLVLTQHNYNNITLDKCVDYNIYGRVGQGFITNVTDSAANSSYLADGGLAILDTSGAIDVFVVQGSYGLNYYKVNPCEDVNQQFVVSGGNIVGILTSRNETGSEQVENQFYVKLTNSSHRRRRSIGQNVTSCSYVSYGRFCIEPDGSLKMIVPEELKQFVAPLLNITESVLIPNSFNLTVTDEYIQTRMDKVQINCLQYVCGNSLECRKLFQQYGPVCDNILSVVNSVGQKEDMELLSFYSSTKPAGYNAPVFSNISTGDFNISLLLTPPSSPSGRSFIEDLLFTSVETVGLPTDAEYKKCTAGPLGTLKDLICAREYNGLLVLPPIITADMQTMYTASLVGAMAFGGITAAGAIPFATQIQARINHLGITQSLLLKNQEKIAASFNKAIGHMQEGFRSTSLALQQVQDVVNKQSAILTEIMNSLNKNFGAISSVIQDIYAQLDAIQADAQVDRLITGRLSSLSVLASAKQSEYIRVSQQRELATQKINECVKSQSNRYGFCGSGRHVLSIPQNAPNGIVFIHFSYTPESFVNVTAIVGFCVQPANASQYAIVPVNGRGIFIQVNGSYYITARDMYMPRDITAGDVVTLTSCQANYVNVNKTVITTFVEDDDFDFDDELSKWWNDTKHELPDFDDFNYTVPILNISGEIDHIQGVIQGLNDSLINLEELSILKTYIKWPWYVWLAIGFAIIIFILILGWVFFMTGCCGCCCGCFGIIPLMSKCGKKSSYYTTFDNDVVT